European Patent Application EP 4 218 428 A1, published August 2, 2023. Title: COMPOSITION COMPRISING GLUCOSYLATED STEVIA AND HAVING IMPROVED SWEETNESS QUALITY. Applicant: CJ CheilJedang Corporation. The sequence listing filed with the application follows.

SEQUENCE LISTING (1 sequence)

SEQ ID NO: 1 - protein, 734 aa, Lactobacillus mali
MDQMVLETQQWLNKTYGGVSGFGSVTEDGLTGWGTVYGLTRALQHELGITGLVNNFGPTSKQKFNNIAKTIVVGYTGNIAYIIQGGFWCKGITPGEFDGKFSADTASAVTTMKTKAGLADTSSSVDGNFMAALLNMSSFDLLTGGDSKVREMQQQLNHDYLAYTGILPCDGIYQRDTNSALIYALQAEEKISTSVATGAYGATTKKDTPTVKEGTTNNFVRILQWGLYVNNKAYTGAFDGVYDSAVVAAVKEFEETMALDSTDGTSAGVDIFMSLLTSAGNPDRSAIACDTSYQLNATRVATLKNAGYSIVGRYLTGTVGSGTSERAKNLTTDEITAITTGGLKIFPIYQDGASDKEAYFTAAQGKTDGTKAVYAAQDLGFKEGVVIYFAVDADIQAGDIAGSAKVYFEALYDIVTSYGYEVGIYGTRNVSATIISAGLATKAFISDMSTGYSGNLGYSIPDEWAFDQFSEISIGDFAIDKDATTSARETATGSFGVGGESGYGNAEDLAKINTIIDALSQKKNFSYLSGLKIEKTSKEYEIPGFAVDFYVQVKFEASVSEPGDNVGVVYNVSNGKFESDFTDTIAGVVALSDEINKEDINSALTELSSLINNGQIWVEPVTKGSDAGIALHIKSTFDHTLDSGETIELEYEIIIDEIFHKIEVVPTGVPNTTANDYNSLFPNGIKEFVGFSIVAGLATGGIYYVVTAVGATAAVVTTSILALIALLKNNDTGV